European Patent Application EP 4 417 696 A1, published August 21, 2024. Title: Mutant of Corynebacterium glutamicum with enhanced L-lysine productivity and method for preparing L-lysine using the same. Applicant: DAESANG CORPORATION. The sequence listing filed with the application follows.

SEQUENCE LISTING (24 sequences)

SEQ ID NO: 1 - DNA, 1278 bp, Corynebacterium sp.
  source 1..1278: mol_type = genomic DNA
gtggctgaaatcatgcacgtattcgctcgcgaaattctcgactcccgcggtaacccaaccgtcgaggcagaggttttcctggatgacggttcccacggtgtcgcaggtgttccatccggcgcatccaccggcgtccacgaggctcatgagctgcgtgacggtggcgatcgctacctgggcaagggcgttttgaaggcagttgaaaacgtcaacgaagaaatcggcgacgagctcgctggcctagaggctgacgatcagcgcctcatcgacgaagcaatgatcaagcttgatggcaccgccaacaagtcccgcctgggtgcaaacgcaatccttggtgtttccatggctgttgcaaaggctgctgctgattccgcaggcctcccactgttccgctacatcggtggaccaaacgcacacgttcttccagttccaatgatgaacatcatcaacggtggcgctcacgctgactccggtgttgacgttcaggaattcatgatcgctccaatcggtgcagagaccttctctgaggctctccgcaacggcgcggaggtctaccacgcactgaagtccgtcatcaaggaaaagggcctgtccaccggacttggcgatgagggcggcttcgctccttccgtcggctccacccgtgaggctcttgaccttatcgttgaggcaatcgagaaggctggcttcaccccaggcaaggacatcgctcttgctctggacgttgcttcctctgagttcttcaaggacggcacctaccacttcgaaggtggccagcactccgcagctgagatggcaaacgtttacgctgagctcgttgacgcgtacccaatcgtctccatcgaggacccactgcaggaagatgactgggagggttacaccaacctcaccgcaaccatcggcgacaaggttcagatcgttggcgacgacttcttcgtcaccaaccctgagcgcctgaaggagggcatcgctaagaaggctgccaactccatcctggttaaggtgaaccagatcggtaccctcaccgagaccttcgacgctgtcgacatggctcaccgcgcaggctacacctccatgatgtcccaccgttccggtgagaccgaggacaccaccattgctgacctcgcagttgcactcaactgtggccagatcaagactggtgctccagcacgttccgaccgtgtcgcaaagtacaaccagcttctccgcatcgagcagctgcttggcgacgccggcgtctacgcaggtcgcagcgcattcccacgctttcagggctaa

SEQ ID NO: 2 - protein, 425 aa, Corynebacterium sp.
VAEIMHVFAREILDSRGNPTVEAEVFLDDGSHGVAGVPSGASTGVHEAHELRDGGDRYLGKGVLKAVENVNEEIGDELAGLEADDQRLIDEAMIKLDGTANKSRLGANAILGVSMAVAKAAADSAGLPLFRYIGGPNAHVLPVPMMNIINGGAHADSGVDVQEFMIAPIGAETFSEALRNGAEVYHALKSVIKEKGLSTGLGDEGGFAPSVGSTREALDLIVEAIEKAGFTPGKDIALALDVASSEFFKDGTYHFEGGQHSAAEMANVYAELVDAYPIVSIEDPLQEDDWEGYTNLTATIGDKVQIVGDDFFVTNPERLKEGIAKKAANSILVKVNQIGTLTETFDAVDMAHRAGYTSMMSHRSGETEDTTIADLAVALNCGQIKTGAPARSDRVAKYNQLLRIEQLLGDAGVYAGRSAFPRFQG

SEQ ID NO: 3 - DNA, 1278 bp, synthetic construct
  source 1..1278: mol_type = other DNA
atggctgaaatcatgcacgtattcgctcgcgaaattctcgactcccgcggtaacccaaccgtcgaggcagaggttttcctggatgacggttcccacggtgtcgcaggtgttccatccggcgcatccaccggcgtccacgaggctcatgagctgcgtgacggtggcgatcgctacctgggcaagggcgttttgaaggcagttgaaaacgtcaacgaagaaatcggcgacgagctcgctggcctagaggctgacgatcagcgcctcatcgacgaagcaatgatcaagcttgatggcaccgccaacaagtcccgcctgggtgcaaacgcaatccttggtgtttccatggctgttgcaaaggctgctgctgattccgcaggcctcccactgttccgctacatcggtggaccaaacgcacacgttcttccagttccaatgatgaacatcatcaacggtggcgctcacgctgactccggtgttgacgttcaggaattcatgatcgctccaatcggtgcagagaccttctctgaggctctccgcaacggcgcggaggtctaccacgcactgaagtccgtcatcaaggaaaagggcctgtccaccggacttggcgatgagggcggcttcgctccttccgtcggctccacccgtgaggctcttgaccttatcgttgaggcaatcgagaaggctggcttcaccccaggcaaggacatcgctcttgctctggacgttgcttcctctgagttcttcaaggacggcacctaccacttcgaaggtggccagcactccgcagctgagatggcaaacgtttacgctgagctcgttgacgcgtacccaatcgtctccatcgaggacccactgcaggaagatgactgggagggttacaccaacctcaccgcaaccatcggcgacaaggttcagatcgttggcgacgacttcttcgtcaccaaccctgagcgcctgaaggagggcatcgctaagaaggctgccaactccatcctggttaaggtgaaccagatcggtaccctcaccgagaccttcgacgctgtcgacatggctcaccgcgcaggctacacctccatgatgtcccaccgttccggtgagaccgaggacaccaccattgctgacctcgcagttgcactcaactgtggccagatcaagactggtgctccagcacgttccgaccgtgtcgcaaagtacaaccagcttctccgcatcgagcagctgcttggcgacgccggcgtctacgcaggtcgcagcgcattcccacgctttcagggctaa

SEQ ID NO: 4 - protein, 425 aa, synthetic construct
MAEIMHVFAREILDSRGNPTVEAEVFLDDGSHGVAGVPSGASTGVHEAHELRDGGDRYLGKGVLKAVENVNEEIGDELAGLEADDQRLIDEAMIKLDGTANKSRLGANAILGVSMAVAKAAADSAGLPLFRYIGGPNAHVLPVPMMNIINGGAHADSGVDVQEFMIAPIGAETFSEALRNGAEVYHALKSVIKEKGLSTGLGDEGGFAPSVGSTREALDLIVEAIEKAGFTPGKDIALALDVASSEFFKDGTYHFEGGQHSAAEMANVYAELVDAYPIVSIEDPLQEDDWEGYTNLTATIGDKVQIVGDDFFVTNPERLKEGIAKKAANSILVKVNQIGTLTETFDAVDMAHRAGYTSMMSHRSGETEDTTIADLAVALNCGQIKTGAPARSDRVAKYNQLLRIEQLLGDAGVYAGRSAFPRFQG

SEQ ID NO: 5 - DNA, 753 bp, Corynebacterium sp.
  source 1..753: mol_type = genomic DNA
atgaccccagcaaacgaaagtcctatgactaatccattaggttctgcccccaccccagccaagccacttcttgacagtgttcttgatgagctcggtcaagatatcatcagtggcaaggttgctgtcggagataccttcaagctgatggacatcggcgagcgttttggcatttcccgcacagtggcacgcgaagcgatgcgcgctttggagcagctcggtcttgtcgcttcttcacgtcgcattggcattactgttttgccacaggaagagtgggctgtttttgataagtccatcattcgctggcgtctcaatgacgaaggtcagcgtgaaggccagcttcagtctcttaccgagcttcgtattgctattgaaccgattgccgcgcgcagcgttgctcttcacgcgtcaaccgccgagctcgagaaaatccgcgcgctcgcaacagagatgcgtcagttgggtgaatctggtcagggtgcgtcccagcgcttcctcgaagcggacgtcactttccacgagctcatcttgcgttattgccacaatgagatgttcgctgcactgattccgtcgattagcgcggttcttgtcggccgcaccgagctcggcctgcagcctgatctgccggcgcacgaggcgctagacaaccacgataagcttgccgacgccctccttaaccgcgacgccgacgccgcagaaactgcgtcccgaaacatcctcaatgaggtgcgcagcgcgctgggcacgctgaactaa

SEQ ID NO: 6 - protein, 250 aa, Corynebacterium sp.
MTPANESPMTNPLGSAPTPAKPLLDSVLDELGQDIISGKVAVGDTFKLMDIGERFGISRTVAREAMRALEQLGLVASSRRIGITVLPQEEWAVFDKSIIRWRLNDEGQREGQLQSLTELRIAIEPIAARSVALHASTAELEKIRALATEMRQLGESGQGASQRFLEADVTFHELILRYCHNEMFAALIPSISAVLVGRTELGLQPDLPAHEALDNHDKLADALLNRDADAAETASRNILNEVRSALGTLN

SEQ ID NO: 7 - DNA, 753 bp, synthetic construct
  source 1..753: mol_type = other DNA
atgaccccagcaaacgaaagtcctatgactaatccattaggttctgcccccaccccagccaagccacttcttgacagtgttcttgatgagctcggtcaagatatcatcagtggcaaggttgctgtcggagataccttcaagctgatggacatcggcgagcgttttggcatttcccgcacagtggcacgcgaagcgatgcgcgctttggagcagctcggtcttgtcgctttttcacgtcgcattggcattactgttttgccacaggaagagtgggctgtttttgataagtccatcattcgctggcgtctcaatgacgaaggtcagcgtgaaggccagcttcagtctcttaccgagcttcgtattgctattgaaccgattgccgcgcgcagcgttgctcttcacgcgtcaaccgccgagctcgagaaaatccgcgcgctcgcaacagagatgcgtcagttgggtgaatctggtcagggtgcgtcccagcgcttcctcgaagcggacgtcactttccacgagctcatcttgcgttattgccacaatgagatgttcgctgcactgattccgtcgattagcgcggttcttgtcggccgcaccgagctcggcctgcagcctgatctgccggcgcacgaggcgctagacaaccacgataagcttgccgacgccctccttaaccgcgacgccgacgccgcagaaactgcgtcccgaaacatcctcaatgaggtgcgcagcgcgctgggcacgctgaactaa

SEQ ID NO: 8 - protein, 250 aa, synthetic construct
MTPANESPMTNPLGSAPTPAKPLLDSVLDELGQDIISGKVAVGDTFKLMDIGERFGISRTVAREAMRALEQLGLVAFSRRIGITVLPQEEWAVFDKSIIRWRLNDEGQREGQLQSLTELRIAIEPIAARSVALHASTAELEKIRALATEMRQLGESGQGASQRFLEADVTFHELILRYCHNEMFAALIPSISAVLVGRTELGLQPDLPAHEALDNHDKLADALLNRDADAAETASRNILNEVRSALGTLN

SEQ ID NO: 9 - DNA, 30 bp, synthetic construct
  source 1..30: mol_type = other DNA
tgattacgccggcgacttatgggattggat

SEQ ID NO: 10 - DNA, 20 bp, synthetic construct
  source 1..20: mol_type = other DNA
ggcgacttatgggattggat

SEQ ID NO: 11 - DNA, 20 bp, synthetic construct
  source 1..20: mol_type = other DNA
tatgccaacttgggagctaa

SEQ ID NO: 12 - DNA, 19 bp, synthetic construct
  source 1..19: mol_type = other DNA
tgtggcctcctatgccaac

SEQ ID NO: 13 - DNA, 30 bp, synthetic construct
  source 1..30: mol_type = other DNA
ggaggccacaatggctgaaatcatgcacgt

SEQ ID NO: 14 - DNA, 20 bp, synthetic construct
  source 1..20: mol_type = other DNA
atggctgaaatcatgcacgt

SEQ ID NO: 15 - DNA, 19 bp, synthetic construct
  source 1..19: mol_type = other DNA
aactggaagaacgtgtgcg

SEQ ID NO: 16 - DNA, 22 bp, synthetic construct
  source 1..22: mol_type = other DNA
tcatcattggaactggaagaac

SEQ ID NO: 17 - DNA, 28 bp, synthetic construct
  source 1..28: mol_type = other DNA
tgattacgcccatcgaccgcctccgtat

SEQ ID NO: 18 - DNA, 18 bp, synthetic construct
  source 1..18: mol_type = other DNA
catcgaccgcctccgtat

SEQ ID NO: 19 - DNA, 18 bp, synthetic construct
  source 1..18: mol_type = other DNA
cgacaagaccgagctgct

SEQ ID NO: 20 - DNA, 20 bp, synthetic construct
  source 1..20: mol_type = other DNA
cgtgaaaaagcgacaagacc

SEQ ID NO: 21 - DNA, 30 bp, synthetic construct
  source 1..30: mol_type = other DNA
ctttttcacgtcgcattggcattactgttt

SEQ ID NO: 22 - DNA, 20 bp, synthetic construct
  source 1..20: mol_type = other DNA
tcgcattggcattactgttt

SEQ ID NO: 23 - DNA, 20 bp, synthetic construct
  source 1..20: mol_type = other DNA
tgcgcgtatcacgttagttc

SEQ ID NO: 24 - DNA, 19 bp, synthetic construct
  source 1..19: mol_type = other DNA
gcaaacgcagtgcgcgtat